European Patent Specification EP 3 512 965 B1, published March 13, 2024. Title: METHODS OF NUCLEIC ACID SAMPLE PREPARATION FOR ANALYSIS OF CELL-FREE DNA. Applicant: ArcherDX, Inc. The sequence listing filed with the application follows.

SEQUENCE LISTING (8 sequences)

SEQ ID NO: 1 - DNA, 91 bp, Artificial Sequence
  Synthetic Oligonucleotide
  misc_feature (71)..(78): n is a, c, g, or t
aatgatacggcgaccaccgagatctacacatccgtacacactctttccctacacgacgctcttccgatctnnnnnnnnaaccgccaggagt

SEQ ID NO: 2 - DNA, 13 bp, Artificial Sequence
  Synthetic Oligonucleotide
ctcctggcggttt

SEQ ID NO: 3 - DNA, 26 bp, Artificial Sequence
  Synthetic Oligonucleotide
aatgatacggcgaccaccgagatcta

SEQ ID NO: 4 - DNA, 28 bp, Artificial Sequence
  Synthetic Oligonucleotide
atgatacggcgaccaccgagatctacac

SEQ ID NO: 5 - DNA, 61 bp, Artificial Sequence
  Synthetic Oligonucleotide
  misc_feature (41)..(48): n is a, c, g, or t
ccatctcatccctgcgtgtctccgactcagctaaggtaacnnnnnnnngctcttccgatct

SEQ ID NO: 6 - DNA, 13 bp, Artificial Sequence
  Synthetic Oligonucleotide
gatcggaagagct

SEQ ID NO: 7 - DNA, 20 bp, Artificial Sequence
  Synthetic Oligonucleotide
ccatctcatccctgcgtgtc

SEQ ID NO: 8 - DNA, 30 bp, Artificial Sequence
  Synthetic Oligonucleotide
ccatctcatccctgcgtgtctccgactcag